European Patent Application EP 4 755 921 A1, published June 10, 2026. Title: 含有GPRC5D抗体的嵌合抗原受体及其应用. Applicant: 深圳市三启生物技术有限公司. Application CN. The sequence listing filed with the application follows.

SEQUENCE LISTING (35 sequences)

SEQ ID NO: 1 - protein, 9 aa, synthetic construct
GYSITSDYA

SEQ ID NO: 2 - protein, 7 aa, synthetic construct
ISYSGSA

SEQ ID NO: 3 - protein, 16 aa, synthetic construct
ARGGIAGRGRWGAMDY

SEQ ID NO: 4 - protein, 6 aa, synthetic construct
QNVGTN

SEQ ID NO: 5 - protein, 9 aa, synthetic construct
QQYKSYPLT

SEQ ID NO: 6 - protein, 123 aa, synthetic construct
QVQLQESGPGLVKPSETLSLTCTVSGYSITSDYAWNWIRQPPGKGLEWMGYISYSGSATYSPSLKSRITISRDTSKNQFSLKLSSVTAADTAVYYCARGGIAGRGRWGAMDYWGQGTTVTVSS

SEQ ID NO: 7 - protein, 107 aa, synthetic construct
DIQMTQSPSSLSASVGDRVTITCKASQNVGTNVAWYQQKPGQSPKALIYSASYRDSGVPDRFSGSGSGTDFTLTISSLQPEDFATYYCQQYKSYPLTFGQGTRLEIK

SEQ ID NO: 8 - protein, 245 aa, synthetic construct
DIQMTQSPSSLSASVGDRVTITCKASQNVGTNVAWYQQKPGQSPKALIYSASYRDSGVPDRFSGSGSGTDFTLTISSLQPEDFATYYCQQYKSYPLTFGQGTRLEIKGGGGSGGGGSGGGGSQVQLQESGPGLVKPSETLSLTCTVSGYSITSDYAWNWIRQPPGKGLEWMGYISYSGSATYSPSLKSRITISRDTSKNQFSLKLSSVTAADTAVYYCARGGIAGRGRWGAMDYWGQGTTVTVSS

SEQ ID NO: 9 - protein, 119 aa, synthetic construct
QVKLEESGGGLVQAGRSLRLSCAASEHTFSSHVMGWFRQAPGKERESVAVIGWRDISTSYADSVKGRFTISRDNAKKTLYLQMNSLKPEDTAVYYCAARRIDAADFDSWGQGTQVTVSS

SEQ ID NO: 10 - protein, 389 aa, synthetic construct
DIQMTQSPSSLSASVGDRVTITCKASQNVGTNVAWYQQKPGQSPKALIYSASYRDSGVPDRFSGSGSGTDFTLTISSLQPEDFATYYCQQYKSYPLTFGQGTRLEIKGGGGSGGGGSGGGGSQVQLQESGPGLVKPSETLSLTCTVSGYSITSDYAWNWIRQPPGKGLEWMGYISYSGSATYSPSLKSRITISRDTSKNQFSLKLSSVTAADTAVYYCARGGIAGRGRWGAMDYWGQGTTVTVSSGGGGSGGGGSGGGGSGGGGSGGGGSQVKLEESGGGLVQAGRSLRLSCAASEHTFSSHVMGWFRQAPGKERESVAVIGWRDISTSYADSVKGRFTISRDNAKKTLYLQMNSLKPEDTAVYYCAARRIDAADFDSWGQGTQVTVSS

SEQ ID NO: 11 - protein, 45 aa, synthetic construct
TTTPAPRPPTPAPTIASQPLSLRPEACRPAAGGAVHTRGLDFACD

SEQ ID NO: 12 - protein, 120 aa, synthetic construct
WRRKRKEKQSETSPKEFLTIYEDVKDLKTRRNHEQEQTFPGGGSTIYSMIQSQSSAPTSQEPAYTLYSLIQPSRKSGSRKRNHSPSFNSTIYEVIGKSQPKAQNPARLSRKELENFDVYS

SEQ ID NO: 13 - protein, 112 aa, synthetic construct
RVKFSRSADAPAYKQGQNQLYNELNLGRREEYDVLDKRRGRDPEMGGKPRRKNPQEGLYNELQKDKMAEAYSEIGMKGERRRGKGHDGLYQGLSTATKDTYDALHMQALPPR

SEQ ID NO: 14 - protein, 21 aa, synthetic construct
MALPVTALLLPLALLLHAARP

SEQ ID NO: 15 - protein, 574 aa, synthetic construct
MALPVTALLLPLALLLHAARPDIQMTQSPSSLSASVGDRVTITCKASQNVGTNVAWYQQKPGQSPKALIYSASYRDSGVPDRFSGSGSGTDFTLTISSLQPEDFATYYCQQYKSYPLTFGQGTRLEIKGGGGSGGGGSGGGGSQVQLQESGPGLVKPSETLSLTCTVSGYSITSDYAWNWIRQPPGKGLEWMGYISYSGSATYSPSLKSRITISRDTSKNQFSLKLSSVTAADTAVYYCARGGIAGRGRWGAMDYWGQGTTVTVSSTTTPAPRPPTPAPTIASQPLSLRPEACRPAAGGAVHTRGLDFACDSNLFVASWIAVMIIFRIGMAVAIFCCFFLPSWRRKRKEKQSETSPKEFLTIYEDVKDLKTRRNHEQEQTFPGGGSTIYSMIQSQSSAPTSQEPAYTLYSLIQPSRKSGSRKRNHSPSFNSTIYEVIGKSQPKAQNPARLSRKELENFDVYSRVKFSRSADAPAYKQGQNQLYNELNLGRREEYDVLDKRRGRDPEMGGKPRRKNPQEGLYNELQKDKMAEAYSEIGMKGERRRGKGHDGLYQGLSTATKDTYDALHMQALPPR

SEQ ID NO: 16 - protein, 718 aa, synthetic construct
MALPVTALLLPLALLLHAARPDIQMTQSPSSLSASVGDRVTITCKASQNVGTNVAWYQQKPGQSPKALIYSASYRDSGVPDRFSGSGSGTDFTLTISSLQPEDFATYYCQQYKSYPLTFGQGTRLEIKGGGGSGGGGSGGGGSQVQLQESGPGLVKPSETLSLTCTVSGYSITSDYAWNWIRQPPGKGLEWMGYISYSGSATYSPSLKSRITISRDTSKNQFSLKLSSVTAADTAVYYCARGGIAGRGRWGAMDYWGQGTTVTVSSGGGGSGGGGSGGGGSGGGGSGGGGSQVKLEESGGGLVQAGRSLRLSCAASEHTFSSHVMGWFRQAPGKERESVAVIGWRDISTSYADSVKGRFTISRDNAKKTLYLQMNSLKPEDTAVYYCAARRIDAADFDSWGQGTQVTVSSTTTPAPRPPTPAPTIASQPLSLRPEACRPAAGGAVHTRGLDFACDSNLFVASWIAVMIIFRIGMAVAIFCCFFLPSWRRKRKEKQSETSPKEFLTIYEDVKDLKTRRNHEQEQTFPGGGSTIYSMIQSQSSAPTSQEPAYTLYSLIQPSRKSGSRKRNHSPSFNSTIYEVIGKSQPKAQNPARLSRKELENFDVYSRVKFSRSADAPAYKQGQNQLYNELNLGRREEYDVLDKRRGRDPEMGGKPRRKNPQEGLYNELQKDKMAEAYSEIGMKGERRRGKGHDGLYQGLSTATKDTYDALHMQALPPR

SEQ ID NO: 17 - DNA, 8741 bp, synthetic construct
  source 1..8741: mol_type = other DNA
ggcttctgaggcggttaattaaaataaaactagagcgggcccggtactaaccaaactggatctctgctgtccctgtaataaacccgaaaattttgaatttttgtaatttgtttttgtaattctttagtttgtatgtctgttgctattatgtctactattctttcccctgcactgtaccccccaatccccccttttcttttaaaattgtggatgaatactgccatttgtctgcagagcggccgcgtcgagataacttcgtataatgtatgctatacgaagttatgttttgttactttatagaagaaattttgagtttttgtttttttttaataaataaataaacataaataaattgtttgttgaatttattattagtatgtaagtgtaaatataataaaacttaatatctattcaaattaataaataaacctcgatatacagaccgataaaacacatgcgtcaattttacgcatgattatctttaacgtacgtcacaatatgattatctttctagggttaaagagctccagcttttgttccctttagtgagggttaatttcgagcttggcgtaatcatggtcatagctgtttcctgtgtgaaattgttatccgctcacaattccacacaacatacgagccggaagcataaagtgtaaagcctggggtgcctaatgagtgagctaactcacattaattgcgttgcgctcactgcccgctttccagtcgggaaacctgtcgtgccagctgcattaatgaatcggccaacgcgcggggagaggcggtttgcgtattgggcgctcttccgcttcctcgctcactgactcgctgcgctcggtcgttcggctgcggcgagcggtatcagctcactcaaaggcggtaatacggttatccacagaatcaggggataacgcaggaaagaacatgtgagcaaaaggccagcaaaaggccaggaaccgtaaaaaggccgcgttgctggcgtttttccataggctccgcccccctgacgagcatcacaaaaatcgacgctcaagtcagaggtggcgaaacccgacaggactataaagataccaggcgtttccccctggaagctccctcgtgcgctctcctgttccgaccctgccgcttaccggatacctgtccgcctttctcccttcgggaagcgtggcgctttctcatagctcacgctgtaggtatctcagttcggtgtaggtcgttcgctccaagctgggctgtgtgcacgaaccccccgttcagcccgaccgctgcgccttatccggtaactatcgtcttgagtccaacccggtaagacacgacttatcgccactggcagcagccactggtaacaggattagcagagcgaggtatgtaggcggtgctacagagttcttgaagtggtggcctaactacggctacactagaagaacagtatttggtatctgcgctctgctgaagccagttaccttcggaaaaagagttggtagctcttgatccggcaaacaaaccaccgctggtagcggtggtttttttgtttgcaagcagcagattacgcgcagaaaaaaaggatctcaagaagatcctttgatcttttctacggggtctgacgctcagtggaacgaaaactcacgttaagggattttggtcatgagattatcaaaaaggatcttcacctagatccttttaaattaaaaatgaagttttaaatcaatctaaagtatatatgagtaaacttggtctgacagttaccaatgcttaatcagtgaggcacctatctcagcgatctgtctatttcgttcatccatagttgcctgactccccgtcgtgtagataactacgatacgggagggcttaccatctggccccagtgctgcaatgataccgcgagacccacgctcaccggctccagatttatcagcaataaaccagccagccggaagggccgagcgcagaagtggtcctgcaactttatccgcctccatccagtctattaattgttgccgggaagctagagtaagtagttcgccagttaatagtttgcgcaacgttgttgccattgctacaggcatcgtggtgtcacgctcgtcgtttggtatggcttcattcagctccggttcccaacgatcaaggcgagttacatgatcccccatgttgtgcaaaaaagcggttagctccttcggtcctccgatcgttgtcagaagtaagttggccgcagtgttatcactcatggttatggcagcactgcataattctcttactgtcatgccatccgtaagatgcttttctgtgactggtgagtactcaaccaagtcattctgagaatagtgtatgcggcgaccgagttgctcttgcccggcgtcaatacgggataataccgcgccacatagcagaactttaaaagtgctcatcattggaaaacgttcttcggggcgaaaactctcaaggatcttaccgctgttgagatccagttcgatgtaacccactcgtgcacccaactgatcttcagcatcttttactttcaccagcgtttctgggtgagcaaaaacaggaaggcaaaatgccgcaaaaaagggaataagggcgacacggaaatgttgaatactcatactcttcctttttcaatattattgaagcatttatcagggttattgtctcatgagcggatacatatttgaatgtatttagaaaaataaacaaataggggttccgcgcacatttccccgaaaagtgccacctaaattgtaagcgttaatattttgttaaaattcgcgttaaatttttgttaaatcagctcattttttaaccaataggccgaaatcggcaaaatcccttataaatcaaaagaatagaccgagatagggttgagtgttgttccagtttggaacaagagtccactattaaagaacgtggactccaacgtcaaagggcgaaaaaccgtctatcagggcgatggcccactacgtgaaccatcaccctaatcaagttttttggggtcgaggtgccgtaaagcactaaatcggaaccctaaagggagcccccgatttagagcttgacggggaaagccggcgaacgtggcgagaaaggaagggaagaaagcgaaaggagcgggcgctagggcgctggcaagtgtagcggtcacgctgcgcgtaaccaccacacccgccgcgcttaatgcgccgctacagggcgcgtcccattcgccattcaggctgcgcaactgttgggaagggcgatcggtgcgggcctcttcgctattacgccagctggcgaaagggggatgtgctgcaaggcgattaagttgggtaacgccagggttttcccagtcacgacgttgtaaaacgacggccagtgaattgtaatacgactcactatagggcgaattgggtaccttaaccctagaaagatagtctgcgtaaaattgacgcatgcattcttgaaatattgctctctctttctaaatagcgcgaatccgtcgctgtgcatttaggacatctcagtcgccgcttggagctcccgtgaggcgtgcttgtcaatgcggtaagtgtcactgattttgaactataacgaccgcgtgagtcaaaatgacgcatgattatcttttacgtgacttttaagatttaactcatacgataattatattgttatttcatgttctacttacgtgataacttattatatatatattttcttgttatagatatccagacatgataagatacattgatgagtttggacaaaccacaactagaatgcagtgaaaaaaatgctttatttgtgaaatttgtgatgctattgctttatttgtaaccattataagctgcaataaacaagttctatcaggcaccgggcttgcgggtcatgcaccaggtgcgcggtccttcgggcacctcgacgtcggcggtgacggtgaagccgagccgctcgtagaaggggaggttgcggggcgcggaggtctccaggaaggcgggcaccccggcgcgctcggccgcctccactccggggagcacgacggcgctgcccagacccttgccctggtggtcgggcgagacgccgacggtggccaggaaccacgcgggctccttgggccggtgcggcgccaggaggccttccatctgttgctgcgcggccagccgggaaccgctcaactcggccatgcgcgggccgatctcggcgaacaccgcccccgcttcgacgctctccggcgtggtccagaccgccaccgcggcgccgtcgtccgcgacccacaccttgccgatgtcgagcccgacgcgcgtgaggaagagttcttgcagctcggtgacccgctcgatgtggcggtccgggtcgacggtgtggcgcgtggcggggtagtcggcgaacgcggcggcgagggtgcgtacggcccgggggacgtcgtcgcgggtggcgaggcgcaccgtgggcttgtactcggtcatgaattccgaaaggcccggagatgaggaagaggagaacagcgcggcagacgtgcgcttttgaagcgtgcagaatgccgggcctccggaggaccttcgggcgcccgccccgcccctgagcccgcccctgagcccgcccccggacccaccccttcccagcctctgagcccagaaagcgaaggagcaaagctgctattggccgctgccccaaaggcctacccgcttccattgctcagcggtgctgtccatctgcacgagactagtgagacgtgctacttccatttgtcacgtcctgcacgacgcgagctgcggggcgggggggaacttcctgactaggggaggagtagaaggtggcgcgaaggggccaccaaagaacggagccggttggcgcctaccgggggatgtggaatgtgtgcgaggccagaggccacttgtgtagcgccaagtgcccagcggggctgctaaagcgcatgctccagactgccttgggaaaagcgcctcccctacccggtagatatcataacttcgtataatgtatgctatacgaagttatgcggccctcgaggtcgacattgattattgactagttattaatagtaatcaattacggggtcattagttcatagcccatatatggagttccgcgttacataacttacggtaaatggcccgcctggctgaccgcccaacgacccccgcccattgacgtcaataatgacgtatgttcccatagtaacgccaatagggactttccattgacgtcaatgggtggactatttacggtaaactgcccacttggcagtacatcaagtgtatcatatgccaagtacgccccctattgacgtcaatgacggtaaatggcccgcctggcattatgcccagtacatgaccttatgggactttcctacttggcagtacatctacgtattagtcatcgctattaccatgggtcgaggtgagccccacgttctgcttcactctccccatctcccccccctccccacccccaattttgtatttatttattttttaattattttgtgcagcgatgggggcggggggggggggggcgcgcgccaggcggggcggggcggggcgaggggcggggcggggcgaggcggagaggtgcggcggcagccaatcagagcggcgcgctccgaaagtttccttttatggcgaggcggcggcggcggcggccctataaaaagcgaagcgcgcggcgggcgggagtcgctgcgttgccttcgccccgtgccccgctccgcgccgcctcgcgccgcccgccccggctctgactgaccgcgttactcccacaggtgagcgggcgggacggcccttctcctccgggctgtaattagcgcttggtttaatgacggctcgtttcttttctgtggctgcgtgaaagccttaaagggctccgggagggccctttgtgcgggggggagcggctcggggggtgcgtgcgtgtgtgtgtgcgtggggagcgccgcgtgcggcccgcgctgcccggcggctgtgagcgctgcgggcgcggcgcggggctttgtgcgctccgcgtgtgcgcgaggggagcgcggccgggggcggtgccccgcggtgcgggggggctgcgaggggaacaaaggctgcgtgcggggtgtgtgcgtgggggggtgagcagggggtgtgggcgcggcggtcgggctgtaacccccccctgcacccccctccccgagttgctgagcacggcccggcttcgggtgcggggctccgtgcggggcgtggcgcggggctcgccgtgccgggcggggggtggcggcaggtgggggtgccgggcggggcggggccgcctcgggccggggagggctcgggggaggggcgcggcggccccggagcgccggcggctgtcgaggcgcggcgagccgcagccattgccttttatggtaatcgtgcgagagggcgcagggacttcctttgtcccaaatctggcggagccgaaatctgggaggcgccgccgcaccccctctagcgggcgcgggcgaagcggtgcggcgccggcaggaaggaaatgggcggggagggccttcgtgcgtcgccgcgccgccgtccccttctccatctccagcctcggggctgccgcagggggacggctgccttcgggggggacggggcagggcggggttcggcttctggcgtgtgaccggcggctctagagcctctgctaaccatgttcatgccttcttctttttcctacagctcctgggcaacgtgctggttgttgtgctgtctcatcattttggcaaagaattcctcgacggtatcgataagctatcacaagtttgtacattcgaaggatccacgcgtgccaccatggccctgcctgtgaccgccctgctgctgcccctggccctgctgctgcatgccgccaggcctgatattcagatgacacagtctccttcatccctgagcgcttctgtgggcgatagagtgacaattacctgtaaggccagtcagaatgtgggcaccaatgtggcctggtaccagcagaagcccggacagagccctaaggccctgatctatagcgccagctacagggacagcggcgtgcctgacaggttttccggcagcggcagcggcaccgacttcaccctgaccatttcttccctgcagcctgaggatttcgccacctattactgccagcagtacaagagctatcccctgacctttggccaggggacccggctggaaatcaagggcggcggcggcagcggagggggcggctccgggggcggcggcagccaggtgcagctgcaggagagcgggcctggcctggtgaagccctctgagaccctgagcctgacatgcaccgtgagcgggtactccattacctccgactacgcctggaactggatcagacagcctcccggcaagggcctggagtggatgggctacatcagctacagcggcagcgccacctacagcccctctctgaagtctcggattaccatctccagggacacatccaagaaccagtttagcctgaagctgtctagcgtgacagccgccgataccgccgtgtactactgtgccagaggcggcatcgccggcagaggcaggtggggcgccatggactactggggacagggcaccaccgtgaccgtgagctccacaaccaccccagccccaaggcctcccacacccgctcccaccatcgcctcccagcccctgagcctgagaccagaggcctgcagacccgccgccggcggcgccgtgcacaccagaggcctggacttcgcctgcgattccaacctgttcgtggcctcctggatcgccgtgatgattatctttcggatcggcatggccgtggccatcttttgttgctttttcttcccctcttggcgccgcaagaggaaggagaagcagtccgagaccagccccaaggagttcctgaccatctacgaggatgtgaaggacctgaaaacccggaggaatcacgagcaggagcagacattccccggcggcggctccaccatctacagcatgatccagagccagagcagcgcccccacctctcaggagcccgcctacactctgtactctctgatccagcccagcagaaagtccggctccagaaagagaaaccattctccatcttttaatagtacaatctatgaagtgattggaaaaagccagccaaaggcccagaaccctgctcgtctgtctagaaaagaattagagaattttgatgtgtatagcagagtgaaattctctaggtctgctgacgctcctgcctataagcagggccagaatcagctgtataatgagctgaatctgggaaggagagaagaatatgatgtgctggataaaagaaggggcagagatcctgagatgggcggaaaacctagaagaaagaatcctcaggaaggcctgtataatgaactgcagaaggataaaatggctgaagcctatagcgagattggcatgaaaggcgaaagaagaagaggcaagggccatgatggcctgtatcagggactgagtacagccactaaagatacatatgacgccctgcacatgcaggccctgccacctagatgaatgcatgctagcctcgactgtgccttctagttgccagccatctgttgtttgcccctcccccgtgccttccttgaccctggaaggtgccactcccactgtcctttcctaataaaatgaggaaattgcatcgcattgtctgagtaggtgtcattctattctggggggtggggtggggcaggacagcaagggggaggattgggaagacaatagcaggcatgctggggatgcggtgggctctat

SEQ ID NO: 18 - protein, 31 aa, synthetic construct
SNLFVASWIAVMIIFRIGMAVAIFCCFFFPS

SEQ ID NO: 19 - protein, 31 aa, synthetic construct
SNLFVASWIAVMIIFRIGMAVAIFCCFFLPS

SEQ ID NO: 20 - protein, 31 aa, synthetic construct
SNLFVASWIAVMVIFRIGMAVAIFRCLFFPS

SEQ ID NO: 21 - protein, 31 aa, synthetic construct
SNLFVASWIAVMIIFRIGMAVAIFCCLFFPS

SEQ ID NO: 22 - protein, 31 aa, synthetic construct
SNLFVASWIAVMIIFHIGLAIAISHVLFFPS

SEQ ID NO: 23 - protein, 31 aa, synthetic construct
SNLFVASWIAVMIIFHIGMAIAISRCLFFPS

SEQ ID NO: 24 - protein, 252 aa, synthetic construct
QVKLEESGGGLVQAGRSLRLSCAASEHTFSSHVMGWFRQAPGKERESVAVIGWRDISTSYADSVKGRFTISRDNAKKTLYLQMNSLKPEDTAVYYCAARRIDAADFDSWGQGTQVTVSSGGGGSGGGGSGGGGSEVQLVESGGGLVQAGGSLRLSCAASGRTFTMGWFRQAPGKEREFVAAISLSPTLAYYAESVKGRFTISRDNAKNTVVLQMNSLKPEDTALYYCAADRKSVMSIRPDYWGQGTQVTVSS

SEQ ID NO: 25 - protein, 574 aa, synthetic construct
MALPVTALLLPLALLLHAARPDIQMTQSPSSLSASVGDRVTITCKASQNVGTNVAWYQQKPGQSPKALIYSASYRDSGVPDRFSGSGSGTDFTLTISSLQPEDFATYYCQQYKSYPLTFGQGTRLEIKGGGGSGGGGSGGGGSQVQLQESGPGLVKPSETLSLTCTVSGYSITSDYAWNWIRQPPGKGLEWMGYISYSGSATYSPSLKSRITISRDTSKNQFSLKLSSVTAADTAVYYCARGGIAGRGRWGAMDYWGQGTTVTVSSTTTPAPRPPTPAPTIASQPLSLRPEACRPAAGGAVHTRGLDFACDSNLFVASWIAVMIIFRIGMAVAIFCCFFFPSWRRKRKEKQSETSPKEFLTIYEDVKDLKTRRNHEQEQTFPGGGSTIYSMIQSQSSAPTSQEPAYTLYSLIQPSRKSGSRKRNHSPSFNSTIYEVIGKSQPKAQNPARLSRKELENFDVYSRVKFSRSADAPAYKQGQNQLYNELNLGRREEYDVLDKRRGRDPEMGGKPRRKNPQEGLYNELQKDKMAEAYSEIGMKGERRRGKGHDGLYQGLSTATKDTYDALHMQALPPR

SEQ ID NO: 26 - protein, 718 aa, synthetic construct
MALPVTALLLPLALLLHAARPDIQMTQSPSSLSASVGDRVTITCKASQNVGTNVAWYQQKPGQSPKALIYSASYRDSGVPDRFSGSGSGTDFTLTISSLQPEDFATYYCQQYKSYPLTFGQGTRLEIKGGGGSGGGGSGGGGSQVQLQESGPGLVKPSETLSLTCTVSGYSITSDYAWNWIRQPPGKGLEWMGYISYSGSATYSPSLKSRITISRDTSKNQFSLKLSSVTAADTAVYYCARGGIAGRGRWGAMDYWGQGTTVTVSSGGGGSGGGGSGGGGSGGGGSGGGGSQVKLEESGGGLVQAGRSLRLSCAASEHTFSSHVMGWFRQAPGKERESVAVIGWRDISTSYADSVKGRFTISRDNAKKTLYLQMNSLKPEDTAVYYCAARRIDAADFDSWGQGTQVTVSSTTTPAPRPPTPAPTIASQPLSLRPEACRPAAGGAVHTRGLDFACDSNLFVASWIAVMIIFRIGMAVAIFCCFFFPSWRRKRKEKQSETSPKEFLTIYEDVKDLKTRRNHEQEQTFPGGGSTIYSMIQSQSSAPTSQEPAYTLYSLIQPSRKSGSRKRNHSPSFNSTIYEVIGKSQPKAQNPARLSRKELENFDVYSRVKFSRSADAPAYKQGQNQLYNELNLGRREEYDVLDKRRGRDPEMGGKPRRKNPQEGLYNELQKDKMAEAYSEIGMKGERRRGKGHDGLYQGLSTATKDTYDALHMQALPPR

SEQ ID NO: 27 - protein, 31 aa, synthetic construct
SNLFVASWIAVMIIFHIGMAIAISCTVFFPS

SEQ ID NO: 28 - protein, 31 aa, synthetic construct
SNLFVASWIAVMIIFRIGMAVAVSRCLHFPS

SEQ ID NO: 29 - protein, 31 aa, synthetic construct
SNLFVASWIAVMIIFHIGLAIAISRCLFYPS

SEQ ID NO: 30 - protein, 31 aa, synthetic construct
SNLFVASWIAVMVIFRIGMAIAISRALFFPS

SEQ ID NO: 31 - protein, 31 aa, synthetic construct
SNLFVASWIAVMVIFRVGMAVAISRALFFPS

SEQ ID NO: 32 - protein, 31 aa, synthetic construct
SNLFVASWIAVMVIFRIAMAVAISRALFFPS

SEQ ID NO: 33 - protein, 31 aa, synthetic construct
SNLFVASWIAVMVIFRIAMSIAIFRGLFFPS

SEQ ID NO: 34 - protein, 31 aa, synthetic construct
SNLFVASWIAVMVTFRIGMAIAISRALFFPS

SEQ ID NO: 35 - protein, 31 aa, synthetic construct
SNLFVASWIAVMVLFRIAMAIAIIYGLFFPS